European Patent Specification EP 4 139 482 B1, published August 14, 2024. Title: Single step sample preparation for Next Generation Sequencing. Applicant: Medicover GmbH. The sequence listing filed with the application follows.

SEQUENCE LISTING (63 sequences)

SEQ ID NO: 1 - DNA, 26 bp, Artificial Sequence
  E_Sarbeco_F1
acaggtacgttaatagttaatagcgt

SEQ ID NO: 2 - DNA, 22 bp, Artificial Sequence
  E_Sarbeco_R2
atattgcagcagtacgcacaca

SEQ ID NO: 3 - DNA, 19 bp, Artificial Sequence
  RP-F
agatttggacctgcgagcg

SEQ ID NO: 4 - DNA, 20 bp, Artificial Sequence
  RP-R
gagcggctgtctccacaagt

SEQ ID NO: 5 - DNA, 113 bp, Artificial Sequence
  E_sarbeco F1 and E_Sarbeco R2 primers
acaggtacgttaatagttaatagcgtacttctttttcttgctttcgtggtattcttgctagttacactagccatccttactgcgcttcgattgtgtgcgtactgctgcaatat

SEQ ID NO: 6 - DNA, 65 bp, Artificial Sequence
  RP-F and RP-R primers
agatttggacctgcgagcgggttctgacctgaaggctctgcgcggacttgtggagacagccgctc

SEQ ID NO: 7 - DNA, 20 bp, Artificial Sequence
  2019-nCoV_N1-F
gaccccaaaatcagcgaaat

SEQ ID NO: 8 - DNA, 24 bp, Artificial Sequence
  2019-nCoV_Nr-R
tctggttactgccagttgaatctg

SEQ ID NO: 9 - DNA, 20 bp, Artificial Sequence
  2019-nCoV_N2-F
ttacaaacattggccgcaaa

SEQ ID NO: 10 - DNA, 18 bp, Artificial Sequence
  2019-nCov_N2-R
gcgcgacattccgaagaa

SEQ ID NO: 11 - DNA, 22 bp, Artificial Sequence
  2019-nCov_N3-F
gggagccttgaatacaccaaaa

SEQ ID NO: 12 - DNA, 21 bp, Artificial Sequence
  2019-nCov_N3-R
tgtagcacgattgcagcattg

SEQ ID NO: 13 - DNA, 72 bp, Artificial Sequence
  2019-nCoV_N1-F and 2019-nCoV_N1-R primers
gaccccaaaatcagcgaaatgcaccccgcattacgtttggtggaccctcagattcaactggcagtaaccaga

SEQ ID NO: 14 - DNA, 67 bp, Artificial Sequence
  2019-nCoV_N2-F and 2019-nCoV_N2-R primers
ttacaaacattggccgcaaattgcacaatttgcccccagcgcttcagcgttcttcggaatgtcgcgc

SEQ ID NO: 15 - DNA, 72 bp, Artificial Sequence
  2019-nCoV_N3-F and 2019-nCoV_N3-R primers
gggagccttgaatacaccaaaagatcacattggcacccgcaatcctgctaacaatgctgcaatcgtgctaca

SEQ ID NO: 16 - DNA, 55 bp, Artificial Sequence
  2019-nCoV_N1.F
tcgtcggcagcgtcagatgtgtataagagacagctggaccccaaaatcagcgaaa

SEQ ID NO: 17 - DNA, 56 bp, Artificial Sequence
  2019-nCoV_N2.F
tcgtcggcagcgtcagatgtgtataagagacagctgttacaaacattggccgcaaa

SEQ ID NO: 18 - DNA, 58 bp, Artificial Sequence
  2019-nCoV_N3.F
tcgtcggcagcgtcagatgtgtataagagacagctggggagccttgaatacaccaaaa

SEQ ID NO: 19 - DNA, 55 bp, Artificial Sequence
  RP-F.F
tcgtcggcagcgtcagatgtgtataagagacagctgagatttggacctgcgagcg

SEQ ID NO: 20 - DNA, 58 bp, Artificial Sequence
  RdRP_SARS.F
tcgtcggcagcgtcagatgtgtataagagacagctggtgaratggtcatgtgtggcgg

SEQ ID NO: 21 - DNA, 62 bp, Artificial Sequence
  E_Sarbeco.F
tcgtcggcagcgtcagatgtgtataagagacagctgacaggtacgttaatagttaatagcgt

SEQ ID NO: 22 - DNA, 61 bp, Artificial Sequence
  2019-nCoV_N1.R
gtctcgtgggctcggagatgtgtataagagacagccgtctggttactgccagttgaatctg

SEQ ID NO: 23 - DNA, 55 bp, Artificial Sequence
  2019-nCoV_N2.R
gtctcgtgggctcggagatgtgtataagagacagccggcgcgacattccgaagaa

SEQ ID NO: 24 - DNA, 58 bp, Artificial Sequence
  2019-nCoV_N3.R
gtctcgtgggctcggagatgtgtataagagacagccgtgtagcacgattgcagcattg

SEQ ID NO: 25 - DNA, 57 bp, Artificial Sequence
  RP.R
gtctcgtgggctcggagatgtgtataagagacagccggagcggctgtctccacaagt

SEQ ID NO: 26 - DNA, 63 bp, Artificial Sequence
  RdRP_SARSr.R
gtctcgtgggctcggagatgtgtataagagacagccgcaratgttaaasacactattagcata

SEQ ID NO: 27 - DNA, 59 bp, Artificial Sequence
  E_Sarbeco.R
gtctcgtgggctcggagatgtgtataagagacagccgatattgcagcagtacgcacaca

SEQ ID NO: 28 - DNA, 68 bp, Artificial Sequence
  Index primer Forward
aatgatacggcgaccaccgagatctacacgatcgctcgtcggcagcgtcagatgtgtataagagacag

SEQ ID NO: 29 - DNA, 33 bp, Artificial Sequence
  TS-Primer Forward
tcgtcggcagcgtcagatgtgtataagagacag

SEQ ID NO: 30 - DNA, 66 bp, Artificial Sequence
  Index primer Reverse
caagcagaagacggcatacgagattcgccttagtctcgtgggctcggagatgtgtataagagacag

SEQ ID NO: 31 - DNA, 34 bp, Artificial Sequence
  TS-Primer Reverse
gtctcgtgggctcggagatgtgtataagagacag

SEQ ID NO: 32 - DNA, 70 bp, Artificial Sequence
  F-Illu-IndexN509
aatgatacggcgaccaccgagatctacacgatctgactcgtcggcagcgtcagatgtgtataagagacag

SEQ ID NO: 33 - DNA, 70 bp, Artificial Sequence
  F-Illu-IndexN502
aatgatacggcgaccaccgagatctacacctctctattcgtcggcagcgtcagatgtgtataagagacag

SEQ ID NO: 34 - DNA, 70 bp, Artificial Sequence
  F-Illu-IndexN503
aatgatacggcgaccaccgagatctacactatcctcttcgtcggcagcgtcagatgtgtataagagacag

SEQ ID NO: 35 - DNA, 70 bp, Artificial Sequence
  F-Illu-IndexN504
aatgatacggcgaccaccgagatctacacagagtagatcgtcggcagcgtcagatgtgtataagagacag

SEQ ID NO: 36 - DNA, 70 bp, Artificial Sequence
  F-Illu-IndexN505
aatgatacggcgaccaccgagatctacacgtaaggagtcgtcggcagcgtcagatgtgtataagagacag

SEQ ID NO: 37 - DNA, 70 bp, Artificial Sequence
  F-Illu-IndexN506
aatgatacggcgaccaccgagatctacacactgcatatcgtcggcagcgtcagatgtgtataagagacag

SEQ ID NO: 38 - DNA, 70 bp, Artificial Sequence
  F-Illu-IndexN507
aatgatacggcgaccaccgagatctacacaaggagtatcgtcggcagcgtcagatgtgtataagagacag

SEQ ID NO: 39 - DNA, 70 bp, Artificial Sequence
  F-Illu-IndexN508
aatgatacggcgaccaccgagatctacacctaagccttcgtcggcagcgtcagatgtgtataagagacag

SEQ ID NO: 40 - DNA, 66 bp, Artificial Sequence; identical to SEQ ID NO: 30
  R-Illu-IndexN701

SEQ ID NO: 41 - DNA, 66 bp, Artificial Sequence
  R-Illu-IndexN702
caagcagaagacggcatacgagatctagtacggtctcgtgggctcggagatgtgtataagagacag

SEQ ID NO: 42 - DNA, 66 bp, Artificial Sequence
  R-Illu-IndexN713
caagcagaagacggcatacgagattgtgatgagtctcgtgggctcggagatgtgtataagagacag

SEQ ID NO: 43 - DNA, 66 bp, Artificial Sequence
  R-Illu-IndexN704
caagcagaagacggcatacgagatgctcaggagtctcgtgggctcggagatgtgtataagagacag

SEQ ID NO: 44 - DNA, 66 bp, Artificial Sequence
  R-Illu-IndexN705
caagcagaagacggcatacgagataggagtccgtctcgtgggctcggagatgtgtataagagacag

SEQ ID NO: 45 - DNA, 66 bp, Artificial Sequence
  R-Illu-IndexN706
caagcagaagacggcatacgagatcatgcctagtctcgtgggctcggagatgtgtataagagacag

SEQ ID NO: 46 - DNA, 65 bp, Artificial Sequence
  R-Illu-IndexN707
aagcagaagacggcatacgagatgtagagaggtctcgtgggctcggagatgtgtataagagacag

SEQ ID NO: 47 - DNA, 66 bp, Artificial Sequence
  R-Illu-IndexN708
caagcagaagacggcatacgagatcctctctggtctcgtgggctcggagatgtgtataagagacag

SEQ ID NO: 48 - DNA, 66 bp, Artificial Sequence
  R-Illu-IndexN709
caagcagaagacggcatacgagatagcgtagcgtctcgtgggctcggagatgtgtataagagacag

SEQ ID NO: 49 - DNA, 66 bp, Artificial Sequence
  R-Illu-IndexN710
caagcagaagacggcatacgagatcagcctcggtctcgtgggctcggagatgtgtataagagacag

SEQ ID NO: 50 - DNA, 66 bp, Artificial Sequence
  R-Illu-IndexN711
caagcagaagacggcatacgagattgcctcttgtctcgtgggctcggagatgtgtataagagacag

SEQ ID NO: 51 - DNA, 66 bp, Artificial Sequence
  R-Illu-IndexN712
caagcagaagacggcatacgagattcctctacgtctcgtgggctcggagatgtgtataagagacag

SEQ ID NO: 52 - DNA, 15540 bp, Coronavirus
atattaggtttttaccttcccaggtaacaaaccaactaactctcgatctcttgtagatctgttctctaaacgaactttaaaatctgtgtgactgtcacttagctgcatgcttagtgcactcacgcagtttaattataattaattactgtcgttgacaggacacgagtaactcgtctatcttctgcaggttgcttacggtttcgtccgtgttgcagccgatcatcagcataccttggtttcgtccgggtgtgaccgagaggtaagatggagagccttgtccctggtttcaacgagaaaacacacggtccactcagtttgcctgttttacaggttcgtgacgtgcttgtacgtggctttggagactccgtagaggaagctttatcagaggcacgtcaacatcttaaagatggcacttgtggcttagtagaagttgaaaaaggtgttttacctcaacttgaacagccctatgtgttcatcaaacgttctgatgcccgaactgcacctcacggccatgttatggtcgaattagtagcagaactcgatggcattcagtatggtcgtagtggtgagacacttggtgttcttgtccctcatgtaggagaggtaccagttgcttaccgtaaagttcttcttcgtaagaacggtaataaaggagctggtggccatagttacggcgccgatctaaagtcttttgacttaggcgacgagcttggtactgatcctattgaagattttcaagaaaattggaacactaaacatggcagtggtgttacccgtgaactcaagcgtgagcttaacggaggtgcatacactcgctatgtagacaacaacttttgtggcccagatggctaccctcttgagtgcattaaagaccttctggctcgtgctggtaaggcttcttatgctttgtctgaacaattggattttattgacactaagagaggtgtgtactgctgccgtgaacacgagcatgaaattgcttggtacacggaacgctctgaaaagagctatgaattgcagacaccttttgaaattaagttggcaaagaaatttgacaccttcaatggggaatgtccaaattttgtatttcctctaaattcaacaatcaagaccattcaaccaagggttgaaaagaaaaagcttgatggtttcatgggtagaattcgatctgtctatcctgttgcttcaccaaatgaatgcaaccaaatgtgcctctcaattctcatgaagtgtgaccattgtggtgaaacttcatggcagacgggtgattttgttagagccacttgcgaattctgtggtactgaaaatttgactaaagaaggtgccacaacttgtggttacttacctcaaaatgctgttgtaaaactttattgtccagcatgtcataatccagaagtaggacctgagcatagtcttgctgaatatcataatgagtctggtttgaaaaccgttcttcgtaagggtggtcgtaccattgcttatgggggctgtgtgtttgcttatgttggttgctacaacaagtgtgcctattgggttccacgtgctagtgctaacataggctgtaatcacacaggtgttgttggagaaggttctgaaagtctaaacgacaaccttcttgaaatattgcaaaaggagaaagtcaacatcaatattgttggtgactttaaacttaatgaagagattgccattattttggcatctttttctgcctctataagtgcttttgtagaaactgtaaaaggtttggattacaaaacattcaaacaaattgttgaatcctgtggtaactttaaagttacgaagggaaaagcaaagaaaggtgcctggaacataggtgaacaaagttcaatactgagtccgctctatgcgttcccttcagatgctgctcatgttgtacggtctatcttctcacgcacactagaaactgctcaccattctgtgcatgtcttacaaaaggctgctataattatcttagatggaatttcacagtattcattgagactcattgatgctatgatgttcacatctgatttggttactaacaatctagttgtaatggcttacattacgggtggtgttgtacaaatgacttcacagtggctaacaaatatctttggcactgtttatgaaaaacttaaaccggttcttgattggctcgaagagaaattcaaagaaggtatagagtttcttagagacggttgggaaattgttaaatttatctcaacttgtgcttgtgaaatagtcggtggacaaattgtcacctgtgcaaaggaaattaaggagagtgttcagacattctttaagctcgtaaataaatttttggctttgtgtgctgactccatcattattggtggagctaaacttaaagccttgaatttaggtgaaacatttgtcacacactcaaagggattgtacagaaagtgtgttagatccagagaagaaactggcttactcttgcctctgaaagctccaaaagaaattattttcttagagggagaaacacttcccacagaagtgttaacagaggaagttgtcttgaaaactggtgttttacaaccattagaacaacctactaatgaggctgttgaagctccattgattggtacaccagtctgtattaacgggctcatgttgctcgaaattaaagacacagaaaagtactgtgcccttgcacctaatatgatggtaacaaataataccttcacacttaaaggtggtgcaccaacaaaagtcacttttggtgatgacactgtgattgaagtgcagggttacaagagtgtaaacatcacttttgaacttgatgaaaggattgataaagtacttaatgagaagtgctctaattacacagttgaactcggtacagaggtaaacgagttcgcttgtgttgttgctgatgctgtcataaaaactttacaaccagtatctgaactaatcataccactgggcattgatttagacgagtggagtatggctacatactacttgtttgatgagtccggtgaatttaaattgtcttcacatatgtactgttctttctaccctcctgaagatgaaggggaagatgattgtgaagaaggacagtgtgaaccatcaactcaatatgagtatggtactgaggatgactaccaaggtaaacctttggagtttggtgctacttctttttcttcttcttcacaggaagaagaacaagaagaggattggttagaatctgatagtcaggacggccaagagactgcagttgaagaaaataaaataccgagtgttgaagttccacctgttttgcaggtggaatcaacaccagttgttactgaaactagtgaacaaaataatttcacaggttatttaaaattaactgacaatgtcttcattaaaaatgctgacattgtagaagaagctaaaaaggtaaagcctacagtagttgttaatgcagctaatgtttaccttaaacatggaggaggtgttgctggagctttaaataaggcaactaacaacgccatgcaggttgaatctgataagtacataactaccaatgggccactaattgtgggtggtggttgtgttttgagtggacataaccttgctaaaaattgtcttcatgttgttggccctaatgtcaacagaggtgaagacattcaattgcttaaaaatgcttatgaaaatttcaatcaacatgagattttactcgcaccattattatcagctggtatttttggtgctgatcctgtacattctttaagagtttgtgtagaaactgttcacacaaatgtctatctagttgtctttgacaaaaatctctatgacaaacttgtttcaagctttttagagatgaagagtgaaaaacaagtagaacaaaaagttgctgaaaatcctaaagaggaagttaagccattttttactgaaaataaaccttcagttgaacaaagacaacaagctgaagagaagaaaatcaaagccagtattgaagaagttacaactactctagaggagaccaagttccttacagaaaacttgttactttatattgacatcaatggcaatcttcacccagattctgccactcttgttaaagatattgacaccactttcttgaagaaagatgttccatatatagtgggtgatgttattaaagaaggcgctttaactgctgtagttatacctactaaaaaggctggtggcactaccgaaatgcttgctaaagctttaagaaaagtgccaacagataattatataaccacctaccctggtcagggtttaaatggttacactgtagaagaagcaaagacagtgcttaaaaagtgtaaaagtgctttttacattttaccatctattatctctaatgcgaagcaagaaattctaggaactgtttcttggaacttgcgagagatgctcgcacatgcagaagaaacacgtaagttaatgcctgtttgtatggagactaaagctatagtttcaactatacaacgtaagtacaaaggcattaaaatacaggagggtgtggttgattatggtgctagattttacttttacactagtaaaactactgtagcatcacttattaacacacttaacaatctaaatgagactcttgtcacaatgccattaggatatgtgacgcacggtctaaatttagaagaagctgctcggtacatgaggtctctcaaagtaccggctacagtctctgtttcttcaccagatgctgttacagcatataatggttatcttacttcttcttcaaaaacacctgaagaacactttattgaaaccgtttcacttgctggttcctataaagattggtcttattctggacagtctacacaactaggcatagaatttcttaagagaggtgataagagtgtatattacaccagtaatcccactacatttcacctagatggtgaaactatcacctttgataatcttaagacacttctctctttgagagaagtgaggaatattaaagtgtttacaacagtagacaacattaacctccacacgcaagttgtggatatgtctatgacatatggacaacagttcggtccaatttatttggatggagctgatgttactaaaataaaacctcacaattcacatgaaggtaaaacattttatgttttgcctaatgatgataccttacgtgcagaggcttttgagtactaccatacaactgatcctagttttctgggtaggtacatgtcagctttaaaccacactaaaaagtggaaatacccacaagtaaatggtttaacttctataaaatgggcagataacaattgttatcttgctactgcattgttaacaatccaacaaatagagttgaaatttaatccaccagctttacaagacgcctattatagggcaagagctggtgaggctgctaatttttgtgcacttatcctggcctattgtaataagacagtaggtgagttaggtgatgtcagagaaacaatgaattatttgtttcaacatgccaatttagattcttgtaaaagagtcttgaatgtggtgtgtaaaacttgtggacaacagcaaacaactctcaagggtgtagaagctgttatgtatatgggcacactttcttatgaacaacttaagaagggtgtgcagataccttgtatgtgtggtaaacaagctacacaatatctggtacaacaagagtcaccttttgttatgatgtctgcaccgcccgcccaatatgaacttaagcatggtacatttgtttgtgctagtgagtatactggtaattaccagtgtggtcactacaaacatataacttctaaagaaaccttgtattgcatagatggcgctttacttacaaagtcctctgagtataaaggttctattacagatgttttctataaagaaaacagttatacaacaaccataaaaccagttacatacaagttggatggtgttgtttgtacagaaattgatcctaagttggatggttattataagaaagataattcttatttcacagagcaaccaattgatcttgtaccaaaccaaccttacccgaatgcaagctttgacaattttaagtttgtatgtgataataccaaatttgccgatgatttaaatcaattgtctggttataagaaacctgcctcgagagagcttaaggttacattctttcctgacttaaatggtgatgtagtggctattgattataagcactacacaccttcttttaagaaaggagctaaattgctgcataagccaattgtttggcatgttaacaatgcaactaacaaagcaacgtacaaaccaaatatttggtgcatacgttgtctttggagtacaaaaccggttgaaacatcaaattcttttgatgcactggaattaggggacacacagggaatggataatcttgcctgtgaagttctaaaaccagtctctgaagaagtagtggaaaatcctaccatacagaaagacattcttgagtgtaatgtgaaaactaccgaagttgtaggagacattatacttaaaccggcaagtgatggtctaaaaattacaaaagaggttggtcatacagacctaatggctgcttatgttgacaattcaagtcttactattaagaaacctaatgaattatccagagtattaggtttgaaaactttagccactcatggcttggctgctattaatagtgttccttgggacactatagctaattatgttaagcctttccttaataaggttgttagcacaactactaacatagttacacggtgtctaaaccgtgtttgtactaattatatgccttatttgtttactttattgctacaattgtgtacttttactaaaagtacaaattctagaataagagcatctatgccaaccactatagcaaagaatactgttaaaagtgttggtaaattttgtatagaggcttcatttaattatttgaagtcacctaatttttctaaattgataaatattgtaatttggtttttattattaagtgtttgcctaggttctttaatctattcaactgctgctttaggtgtcttaatgtctaatttaggcatgccttcttattgtactgtttacagagaaggttatttgaactctactaatgtcactactgcaacctactgcactggttctataccttgtagtgtttgtcttagtggtttagattctttggatacttacccatccttagaaactatacaaattaccatttcgtcttttaaatgggatttaactgcttttggtctagttgcagagtggtttttggcatatattctttttactaggttcttttatgtacttggattggctgcaatcatgcaattgtttttcagctattttgcagtacattttattagtaattcttggcttatgtggttaataattaatcttgtacaaatggccccaatttcagctatggttagaatgtatattttctttgcatcattttattatgtatggaaaagttatgtgcatgttgtagatggttgtacttcatcaacttgtatgatgtgttataaacgtaatagagcaacaagagttgaatgtacaactattgttaatggtgttagaaggtccttttatgtctatgctaatggaggtaaaggcttttgcaaactacataactggaattgtattaattgtgatacattctgtgctggtagtacatttattagtgacgaagttgctagagacttatcactacagtttaaaagaccaataaatcctactgaccagtcttcctatattgttgatagtgttacagtgaagaatggttccatccatctttactttgataaggctggtcaaaagacttatgaaagacattctctctctcattttgttaacttagacaatctgagagctaataacactaagggttcattgcctattaatgttatagtttttgatggtaaatcaaaatgtgaagaatcatctgctaaatcagcgtctgtttattatagtcagcttatgtgtcaacctatactgttactggaccaggcattagtgtctgatgttggtgacagtgcagaagttgcagttaagatgtttgatgcttatgttaatatattttcatcaactttcaatgttccaatggaaaaactcaaagcattagttgcgactgcagaagctgaacttgcaaagaatgtgtctttagacaacgtcttatctacttttatttcagcagctcgtcaagggtttgttgattcagatgtagaaactaaagatgttgttgaatgtcttaaattgtcacaccaatctgacatagaagttacaggtgacagttgtaacaattacatgctcacttataacaaagttgaaaacatgacacctcgggatcttggtgcttgtattgattgtagtgcacgtcatatcaatgcacaggtggcaaaaagtcataacatagctttgatttggaatgttaaagatttcatgtcattgtctgaacaactacgaaaacaaatacgcagtgctgctaagaagaataacttgccttttagattgacatgtgcaaccactagacaagttgttaatgttgttacaacaaaaatagcacttaagggtggtaaaattgttaacaactggttgaagcagctgattaaggttacacttgtgtttcttttcatcactgttatcttctatttaataacacctgttcatgtcatgtttaaacacaatgacttttcaagtgaaattataggatacaaggctattgatggtggtgtcactcgtgacatagcgtcaacagatacttgttttgctaacaaacatgctgactttgactcttggtttagtcagcgcggtggtagttatactaatgataaagcttgcccattggtagcagctgttatcacaagggaagttggctttgttgtgcccggtttgcctggcacaatattacgcacaattaatggtgattttttgcattttcttcctagagtgtttagtgcggtaggtaacatttgttacactccttctaaacttatagagtacactgactttgcaacatcggcatgcgttttagctgctgaatgtaccatttttaaagatgcttctggtaaaccagtaccttattgttatgatactaatgtactagaaggttctgttgcgtatgaaagtctccgccctgacacacgctatgtgctcatggacggttctataattcaattccctaacacttaccttgaaggttctgttagagtagtaacaacttttgattcagagtattgtagacatggtacttgcgaaagatcagaggctggcatttgtgtatctactagtggtagatgggtacttaataatgattattacagatccttgccaggagttttttgtggtgtagatgctgtgaatttacttactaatatgttcacgccattaattcaacctattggtgctttggacatatctgcatctattgtagcaggtggtgttgtagctattatagtaacttgtctagcctactacttcatgaggtttagaagagcttttggtgaatacagtcatgtagttgcctttaacactctactattctttatgtcattcactgtactctgtttaacaccagtctattcattcttacctggtgtttattctgttatttacttgtacttgacattttatcttactaatgatgtttctttcttagcacatatccaatggatggttatgttcacacccttagtgcctttctggatgacaattgtttatgtcatttgcatttccacaaagcatttttattggttctttagtaactacctaaagagacgtgtagtctttaatggtgtttcctttagtacatttgaggaggctgcattatgtacctttttgttaaataaagaaatgtatctgaaattgcgtagtgatgtacttctacctcttacgcaatacaatagatatttagctctttataataagtacaagtattttagtggggccatggacactaccagttatagagaagcagcttgctgtcatctggctaaggctataaatgatttcagtaattcaggttctgatgtcctctaccaaccaccacaaacttcaatcacatcagcggttttgcagagtggttttagaaaaatggcattcccatctggtaaagttgaaggttgcatggtacaagttacttgtggtaccactacacttaatggtctttggcttgatgatgtagtttactgtccacgacatgtgatctgcacttctgaagacatgctcaatcctaattatgaagatttacttatacgtaaatctaaccataattttttagttcaggctggtaatgttcaacttagagttgttggacattctatgcaaaattgtgttcttaagcttaaagtagatacagctaatcctaagacacctaagtataagtttgtgcgcattcaacccggacagactttttcagtattagcctgttacaatggttcaccatctggtgtttaccaatgtgccatgagacctaattttactattaagggttcattccttaatggttcatgtggtagtgttggttttaatatagactatgactgtgtctctttttgttatatgcatcatatggagttaccaacgggagttcatgctggcacagacttagaaggtaccttctacggaccttttgttgacagacagacagcacaagcggctggtactgacacaactattacagttaatgttctagcttggttgtatgcagctgttataaacggagatagatggttccttaataggtttaccacaactctaaacgattttaatcttgtggctatgaagtataattatgaacctctaacacaagaccatcttgacatactaggacctctttcagctcaaactggaattgcagtcctagatatgtgtgcttcattaaaagaattattacaaaatggtatgaatggacgtaccatattgggtagtgctttattagaagatgaatttacacctttcgatgttgttagacaatgttcaggtgtcacctttcaaagtgcagtgaaaaggacaatcaagggcacgcaccattggttgttgcttacagttttgacttcactcttagttttagttcagagtactcaatggtctttgttcttctttgtgtatgaaaatgcctttatgccttttgctatgggtattattgctatgtctgcttttgctatgatgtttgtcaaacataagcatgcattcctctgtttgttcctgttaccttctcttgctactgtagcttattttaatatggtctacatgcctgctagttgggtgatgcgtattatgacatggttggatatagttgatactagtttgtctggtttcaagctaaaggactgtgttatgtatgcatcagctgtagtgttattaatcctcatgacagcaagaaccgtatatgatgatggtgctagaagagtttggacacttatgaatgtcctgacactcgtttataaagtttattatggtaatgctttagaccaagctatttccatgtgggctcttataatctctgttacttctaactactcaggtgtagttacaactgtcatgtttttggccagaggtattgtttttatgtgtgttgagtattgtcctatcttctttataactggcaatacactccagtgtataatgctagtttattgtttcttaggttatttctgtacttgttattttggtctcttctgtttactcaaccgctattttaggcttactcttggtgtttatgactatttagtctctacacaagaatttaggtacatgaactctcaggggctcctgccacctaagagtagtattgacgctttcaagcttaacattaaattgttgggcattggaggtaaaccttgtattaaggttgctactgtacagtctaaaatgtctgacgtaaagtgcacatcagtagtgcttctctcagttcttcagcaacttagagtagagtcatcttctaaattgtgggcacagtgtgtacaacttcacaatgatattcttcttgccaaggacactactgaagcttttgagaagatggtttcacttttgtctgttttgctgtccatgcagggtgctgtagacattaacaagttgtgcgaggaaatgctcgacaaccgtgctacccttcaggctattgcttcagaattcagttctttaccttcatatgctgcttatgccactgctcaagaggcttatgagcaggctgtagcaaatggtgattctgaagttgttcttaaaaagttaaagaaatctttgaatgtggctaaatctgagtttgaccgtgatgctgccatgcaacgtaagttggaaaagatggcggatcaggctatgacccaaatgtacaagcaggcaagatctgaggacaagagggcaaaagtaactagtgcaatgcaaactatgcttttcactatgcttagaaaacttgataatgatgcacttaacaacattatcaacaatgcacgtgatggttgtgtaccactcaacatcataccactcacaacagcagcaaaactcatggttgttgtccctgactatggaacctacaagaatacttgtgatggtaacacttttacatatgcatcagcactctgggaaatccagcaagttgttgatgcagatagtaaaattgtgcagcttagtgaaatcaacatggacaactcaccaaatttggcttggcctcttattgttactgctttaagagccaattcagctgtcaaactacagaacaatgagctgagtccagtagcactacgacagatgtcctgtgcggctggtactacacagacagcttgtactgatgacaacgcacttgcctactataacaattctaagggaggtaggtttgtgcttgcattactatcagaccaccaggatctcaaatgggctagattccctaagagtgatggtacaggtactatctatacagaattggaaccaccttgcaggtttgttacagacacacctaaaggacctaaagtgaagtatttgtactttattaagggtcttaacaacctaaatagaggtatggtactgggtagtttggctgccacagtacgtcttcaggctggtaatgcgacagaagtgcctgccaattcaactgtgctttctttttgtgcttttgctgtagacccagctaaagcttacaaagattacctagcaagtggtggacaaccaatcacgaattgtgtgaagatgttgtgtacacacactggtacaggacaggcaatcacggtaacaccagaagccaatatggatcaagaatcctttggtggtgcttcatgctgtctgtattgtagatgccacattgatcatccaaatcctaagggattttgtgacttgaaaggtaagtatgttcaaatacctaccacttgtgttaatgaccctgtggggtttacactcagaaacacagtctgtaccgtctgcggaatgtggaaaggttatggctgtagttgtgatcaactccgcgaacccatgatgcagtctgcggatgcgtcaacgtttttaaacgggtttgcggtgtaagtgcggcccgtcttacaccgtgcggcacaggcactagcactgatgtcgtttatagggcttttgatatttacaacgagaaagttgctggttttgcaaagttcctaaaaactaattgctgtcgcttccaagaaaaggatgaggaaggcaatttattagactcttatttcgtagttaagaggcacacaatgtccaactaccaacatgaagagactatttacaacttggttaaagggtgtccagccgttgctgttcatgactttttcaagtttagagtagatggtgacatggtaccacatatatcacgtcaacgtctaactaaatacacaatggctgatttagtctatgctctacgtcattttgacgagggcaattgtgatacattaaaggaaatacttgtcacatacaaatgttgtgatgacaactatttcaataagaaggattggtatgactttgtagaaaatcctgatgttctacgcgtatacgcgaacctaggtgagcgtgtacgtcaagccttattgaaaactgtgcaattctgcgatgctatgcgcgatgcgggtatcgtaggtgtactgacactagacaatcaggatctgaatgggaattggtacgacttcggagatttcgtacaggtagcaccaggctgcggagtccctattgtggattcatactattctttgctgatgcctattctgacactcacaagggctttggctgctgagtcccatatggacgctgatctcgcgaagccacttattaagtgggatttgctgaaatatgatttcacggaagagagactatgtcttttcgaccgttattttaaatattgggaccagacgtaccatcctaattgtattaattgtttggatgacaggtgtatccttcattgtgcaaactttaatgtgttattttctactgtgtttccacctacgagttttggaccactagtaagaaagatatttgtagatggtgtaccttttgttgtttcaacgggataccatttccgtgagctaggggttgtacataatcaggatgtaaacttacataactcgcgtctcagttttaaggaacttttagtgtacgctgctgatccagctatgcatgctgcctctggcaatttgttgttagacaaacgcactacatgcttttcagtagctgcactaacaaacaatgttgcttttcaaactgtcaaacccggtaattttaataaagacttttatgactttgctgtgtctaaaggcttctttaaggaaggaagttctgttgaattaaaacacttcttctttgctcaggatggcaatgctgctatcagtgattatgactattaccgttataatctgccaacaatgtgtgatattagacaactcctattcgtagttgaggttgtcgataaatattttgattgttacgacggtggctgtatcaatgccaaccaagttatcgttaacaatctggacaaatcagccggtttcccatttaataagtggggtaaggctagactttattatgactcaatgagttatgaggatcaagatgcactgttcgcatacactaagcgtaacgtcatccctacaataactcaaatgaatcttaagtatgccattagtgcaaagaatagagctcgcactgttgctggtgtctctatctgtagtactatgaccaatagacagtttcatcagaaattattaaagtcaatagccgccactagaggagctactgtggtaattggaacaagcaaattttatggtggctggcataacatgttaaaaactgtttacagtgatgtagaaagtcctcaccttatgggttgggactacccaaaatgtgacagagccatgcctaatatgcttagaatcatggcttccctcgttcttgctcgcaaacatagcacttgttgtaacttgtcacaccgtttctatagattagctaatgagtgtgcacaagtattaagtgagatggtcatgtgtggcggctcattatatgtgaaaccaggtggaacatcatccggtgatgccacaactgcttatgctaatagtgtgtttaacatctgtcaagcagtaacagctaatgtaa

SEQ ID NO: 53 - DNA, 10780 bp, Coronavirus
atgcacttctttcaactgatggtaataagattgctgataagtatgtccgcaaccttcaacacagactttacgagtgtctctatagaaatagagacgtagatcaggaattcgtggatgaattttatgcatatttgcgtaagcatttctccatgatgattctttctgatgatgccgtcgtatgctataatagtaattacgcggcacagggtctagtagctagcattaagaactttaaagcagttctttattaccaaaataatgtattcatgtctgaggcaaaatgttggactgagactgaccttactaaaggacctcatgaattttgttctcagcataccatgctagttaaacagggagatgattatgtgtacctgccttatccagatccatccagaatattaggcgcaggctgttttgtcgatgacattgtcaaaacagatggtacacttatgattgaaaggtttgtgtcattagcaattgacgcctatccacttacaaagcaccctaatcaagagtatgctgatgttttccatttatacttacagtatattaggaaattacatgatgagcttactggtcacatgttggacatgtactctgtaatgctaactaatgacaacacctcgaggtactgggaacctgagttttatgaggcaatgtacacaccacacacagttttgcaagctgtaggtgcgtgtgtgttatgcaattcacagacttcacttcgttgcggtgcttgtattaggagacctttcctttgttgcaagtgctgctatgatcacgtcatctcaacatcacataaattagtgttgtctgttaatccctatgtttgcaatgcacccggttgtgatgtcacagacgtaacacaactctatttgggaggtatgagctattactgcaagtcacataaaccacccattagttttccgttgtgtgctaatggtcaggtttttggtttgtacaaaaacacatgtgtgggcagtgataacgtaactgacttcaatgcaatagcgacatgcgactggactaatgctggcgattacatacttgccaacacttgcacagagagactcaaactttttgcagcggaaacgctcaaagctactgaggaaacattcaaactatcttatggtattgccactgttcgtgaagtactgtcagatagagaacttcatctttcatgggaggtaggaaaacctagaccaccattgaatagaaattacgtctttactggttaccgtgtgaccaaaaatagtaaagtacagattggagagtatacctttgaaaaaggtgactatggtgatgctgttgtgtacagaggtactacaacttataaattgaatgttggtgattactttgtgttaacatcacacacagtaatgccactaagtgcaccaacactagtgccacaagagcactatgtgcgaataactggcttataccctacacttaatatctctgatgagttttctagcaatgttgcaaattaccaaaaggtcggcatgcagaagtactccacactccagggaccacctggtactggtaagagtcactttgctattggacttgccctctactacccatctgcccgcatagtgtatacagcttgctctcatgctgctgttgatgcgctatgtgagaaggcattaaaatacttgcctatagataagtgtagtagaattattcctgcacgtgcgcgtgtagagtgttttgacaaattcaaagtgaattcaaccttagaacagtatgttttctgcactgtcaatgcgctgcctgaaactactgctgatatagtggtctttgatgaaatttcaatggccactaattatgatttgagtgttgtcaatgccagactacgtgcaaaacactacgtttacattggtgatccggctcaattacctgcaccacgcacattgctaacaaaaggcacacttgaaccagaatatttcaattcagtgtgcagacttatgaaaacaataggtccagacatgttccttgggacttgtcgtcgttgtcccgctgaaattgttgacacagtgagtgctttagtttatgataataagctaaaagcacacaaagagaagtcagctcaatgcttcaagatgttttacaagggtgtgattacgcatgatgtgtcatccgcaatcaacagaccacaaataggtgtagtaagagaatttcttacgcgcaatccagcttggagaaaagctgtttttatttcaccatataattcacagaatgcagtggcatcaaagattttagggttgcctactcaaactgttgattcttcacagggttctgaatatgactatgtcatattcacacaaaccactgagactgcacactcttgtaatgtaaaccgctttaatgtggccattacaagagcaaagattggcattttgtgcataatgtctgatagagacctttatgacaagcttcaatttatgagtctagaagtaccgcgtcgaaatgtggctactttacaagcagaaaatgtgactggactctttaaggactgtagcaagatcattactggtcttcatccaacacaggcacctacgcatctcagtgttgatactaaattcaagactgaaggactttgtgtcgacataccaggaataccaaaggacatgacctatcgtagactcatctctatgatgggctttaaaatgaattaccaagttaatggttaccctaatatgtttatcacccgtgaagaagctattcgtcacgttcgtgcatggataggctttgatgttgagggttgtcatgcgactagagatgctgtaggaacaaatctaccactccagttagggttttcaacaggtgttaacctagtggctgtaccaactggctatgttgacactgagcacagcacagaatttaccagagttaatgcaaaacctcctccaggtgatcaatttaagcatcttataccacttatgtacaaaggcttgccctggaacgtggtgcgtattaagattgttcaaatgctcagtgatacactgaaaggattatcagacagagttgtgtttgtcctttgggcacatggctttgaacttacatcgatgaagtattttgttaagatcggaccagaaagaacgtgttgtctgtgtgacaaacgcgcgacttgcttctctacttcatctgacacttatgcctgttggaatcactctgtgggctttgactatgtctataacccgtttatgattgatgtccagcagtggggttttacaggtaaccttcaaagtaaccatgatcaacactgccaagtgcatggtaatgcccatgtagctagttgtgatgctatcatgactagatgtcttgcagtccatgagtgctttgttaagcgcgttgattggtctgttgaatacccgattattggagatgaactgaagattaatgccgcatgcagaaaagtacagcatatggttgttaaatctgcattgcttgctgataaattcccagttcttcatgatataggaaacccaaaggctattagatgtgtgccgcagtctgaagtggactggaaattctacgacgctcagccttgcagtgacaaagcttataaaatagaagaactcttctactcatatgccacacatcatgacaagttcacagatggtgtttgcttgttttggaactgtaacgttgatcgttacccggctaatgctattgtgtgtaggtttgatactagagtgctttctaatttaaacctaccaggttgtgatggtggtagtttgtatgttaataagcatgcgttccacactccagcttttgataagagtgcatttacacatttgaaacaactgcctttcttttattactctgacagtccgtgtgagtctcatggtaaacaggttgtgtcagatattgattatgtcccactaaagtctgctacgtgtattacacgatgcaacttaggtggtgccgtttgtagacatcatgcaaacgagtacagacagtacttggatgcatataatatgatgatttctgctggatttagcctttggatttataaacaatttgatacttacaacttgtggaacactttcaccaagttgcagagtttagaaaatgtggcttataatgttatcaacaagggacactttgatggacagaatggtgaagcacctgtgtctatcgttaataatgctgtttacactaagttagatggtgttgatgtggagatctttgaaaataagacaacacttcctgttaatgttgcatttgagctttgggctaaacgtaacattaaaccggtgccagagattaaaatactcaataatttgggtgttgatatcgctgctaatactgttatatgggactacaagagagaagcgccagcgcatgtttctacaataggtgtctgtacaatgactgacattgcaaagaaacctactgagagtgcttgttcatcacttactgtcttatttgatggtagagttgagggacaggtagacctttttagaaacgcccgtaatggtgttttaataacagaaggttcagttaagggcttaacaccttcgaaaggacctgcacaggctagtgtcaacggagtcacattaattggagaatcagtaaaaacacagttcaattactttaagaaagtggatggcattattcagcaattgccagaaacctactttactcaaagcagagacttagaggatttcaagcccagatcacaaatggaaactgatttccttgagctcgctatggatgaattcatagaacgatataagctagatggctatgctttcgagcacatcgtttatggagattttagtcatggacaattaggcggacttcatttattgataggactggccaaaaggtcacaggactcactgttaaagctagaggattttattcctatggatagcacagtgaaaaactacttcataacagatgcgcaaacgggttcatctaagtgtgtatgctctgttatcgaccttttacttgatgactttgttgaaataataaagtcacaagatctttcagtggtttcaaaagtagtcaaagttacgattgattatacagaaatttcatttatgctttggtgtaaagatgggcatgtggaaactttttacccaaaattacaatctagtcaagcatggcaaccaggtgttgctatgcctaatctctataaaatgcagagaatgttactggaaaagtgtgatcttcaaaattatggtgatagtgctatattgcctaaaggcataatgatgaatgtcgcaaagtacactcaactgtgtcagtatttaaatacacttactttagctgtgccctataatatgagagttatacattttggcgcgggctctgataaaggagtagcacctggcacagctgttcttagacagtggttgccaactggtacactacttgtcgattctgatttaaatgattttgtttctgatgcagactcaacattaattggtcattgtgcaaccgtacatacggctaataaatgggatctcattattagcgatatgtatgatcctaagactaaaaatgttacaaaagagaatgattccaaagaaggatttttcacttacatttgtggatttatacagcaaaaattagccctcggaggttccgtagctgtaaagataacagagcattcctggaatgctgatctttataagctcatgggacacttcgcatggtggacagcttttgttactaatgttaatgcttcatcttcagaggctttcttaattggttgtaattatcttggcaaaccacgtgagcagatagatggttatgtcatgcatgcaaattacatattttggaggaacacaaatccaatacaattgtcttcctactcattatttgacatgagtaagtttcctcttaaattaagaggtactgctgttatgtcattaaaagatggacaaatcaatgatatgattttgtctcttcttagtaaaggcagacttattgttagagagaataatagagttattatctctagtgatgttcttgttaacaactaaacgaacatgttgtttttcttgtttcttcagttcgccttagtaaactcccagtgtgttaacttgacaggcagaaccccactcaatcccaattatactaattcttcacaaagaggtgtttattaccctgacacaatttatagatcagacacacttgtgctcagccagggttattttcttccattttattctaatgttagctggtattactcattaacaaccaacaatgctgccacaaagaggactgataatcctatattagatttcaaggacggcatatactttgctgccactgaacactcaaatattatcaggggctggatctttggaacaactcttgacaacacttctcaatctctcttgatagttaacaacgcaacgaatgttattatcaaggtttgtaattttgatttttgttatgatccctaccttagtggttactatcataacaacaaaacatggagcatcagagaatttgctgtctattcttcttatgctaattgtacttttgagtatgtttcgaaatcctttatgttgaacatttctggtaatggtggtctgttcaacactcttagagagtttgttttcagaaatgtcgatgggcatttcaagatttactcaaagtttacaccagtaaatttaaatcgtggcttgcctactggtctctcagtgcttcagccattggttgaattaccagttagcataaatattactaaattcagaacactcctcactattcatagaggagaccctatgcctaataacggctggactgctttttcagctgcttatttcgtgggctatcttaaaccacgtacctttatgctgaaatataatgagaatggcaccattactgatgctgttgattgtgcacttgaccctctttcggagacaaagtgtacgttaaaatctcttactgtccaaaagggcatctatcagacttctaacttccgagtgcaacccactcagtctgtagttagatttcctaatattaccaatgtgtgtccatttcacaaggtttttaatgccacgaggtttccttccgtctatgcgtgggaaagaactaaaatttctgattgcattgcagattacactgttttctacaattcaacttctttttctacttttaaatgttatggtgtttcaccttctaaattgattgatttgtgctttacgagtgtgtatgctgatacatttctcataagattctcagaagtcagacaggtggcaccaggacaaactggtgtcattgctgactataattataaattacctgatgattttacaggttgtgtcatagcttggaacactgccaaacaggatgtaggtaattatttctacaggtctcatcgttctaccaaattgaaaccatttgaaagagatctttcctcagacgagaatggtgtccgtacacttagtacttatgacttcaaccctaatgtaccacttgaataccaagctacaagggttgttgttttgtcatttgagcttctaaatgcaccagctacagtttgtggaccaaaactatccacacaactagtaaaaaatcagtgcgttaatttcaactttaacggactcaagggcactggtgtcttgactgattcttccaagaggtttcagtcattccaacaatttggtaaagatgcgtctgactttattgattcagtacgtgatcctcaaacacttgagatacttgacattacaccttgctcttttggtggtgtcagtgttataacaccaggaacaaacacttctttagaggtggctgttctttaccaagatgttaactgcactgatgtaccaactactatacatgcagaccaactaacacctgcttggcgtatttatgctactggcactaatgtgtttcaaactcaagcaggctgtcttataggagctgaacatgtcaatgcttcttatgagtgtgacatcccaattggtgctggtatttgtgctagctaccatacggcttctatattacgcagtacaagccagaaagctattgtggcttatactatgtcccttggtgctgagaactctatcgcttatgctaacaattctatagccatacctacaaatttttcaattagtgttaccactgaagttatgcctgtatcaatggctaaaacttctgtagattgtactatgtatatctgtggtgactctatagagtgtagcaacttgttgttacaatatggcagtttttgcacacaactaaatcgtgctttaagtgggattgctattgagcaagacaagaacacccaagaggtttttgctcaagttaagcaaatctataaaacaccacctattaaggattttggtggttttaatttttcacagatactacctgacccatctaaacccagcaagaggtcgtttattgaagacttactcttcaataaagtcactcttgctgatgccggttttatcaaacagtacggtgattgtttgggtggtatttctgctagagatttgatttgtgctcaaaagttcaatggacttactgtcttaccaccattgctcacagatgaaatgatcgctgcttatacagctgcattaattagcggcactgccactgctggatggacctttggtgctggtgctgctcttcaaataccatttgccatgcaaatggcttataggtttaatggaattggagttactcagaatgttctctatgagaatcagaaattaatagccaatcagtttaatagtgctattggaaaaatccaagagtctttgacatctacagctagtgcacttggaaaattgcaggatgttgttaaccaaaatgcacaagctttaaacacgcttgttaaacaacttagttccaattttggtgcaatttcaagcgtgttgaatgacattctttcacgccttgacaaagtcgaggctgaggttcagattgataggttgatcacaggtagacttcagagtttacagacgtatgtgactcaacaattaatcagagctgcagaaatcagagcttctgctaatcttgctgcgactaaaatgtccgagtgtgtactaggacaatctaaaagagttgatttttgtggaaaaggttatcacctaatgtcttttccccagtcagcgcctcatggtgttgtcttcttacatgtgacttacattccttcgcaagaaaagaacttcacaacagctcctgccatttgccatgaaggtaaagcacacttcccacgtgaaggtgttttcgtttcgaatggcacacactggtttgtaacacaaaggaacttttatgaacctaaaattataaccactgacaatacatttgtctctggtaactgtgatgttgtaattggaattatcaacaacacagtttatgatcctttacaaccagaacttgattcatttaaggaggagttagataaatattttaaaaatcatacatcacctgatattgatcttggtgatatttctggcattaatgcttctgttgtcaatattcaaaaggaaattgaccgcctcaatgaggttgccagaaatttaaatgaatcactcattgatctccaagaacttggaaaatatgagcaatatatcaaatggccatggtatgtttggctcggcttcattgctggactcattgctatagtcatggttacaatcctgctttgttgcatgacaagttgttgcagttgtctcaagggctgttgttcttgcggatcttgctgtaaatttgatgaagacgactctgagcctgtgctcaaaggagtcaaattacattacacataaacgaacttatggatttgtttatgagaattttcactcttggaactgttactcttaaacaaggtgaaatcaaaggtgctactcctacaaattctgttcgcactactgcaacaataccgatacaagccacactccctttcggatggcttgttgttggcgttgcaattcttgctgtttttcaaagcgcttcaaaaataattacactcaaaaagagatggcagttagccctctctaaaggtgttcattttgtttgcaacttgcttctgctgtttttaacagtttattctcacttgttgcttcttgctggtggcttggaagccacttttctctttctttatgcattagcttattgcttgcaaactgtaaattttgtgagaataataatgcgattctggttgtgctggaagtgccgttccaagaatcctttactctatgatgccaactactttctttgttggcatactaattgttatgactattgtataccatacaatagtgtaacctcttcaattgtcatcacatgtggtgatggtactacgaatcccatttctgaggacgactaccaaattggtggttacacggaaaagtgggagtctggtgttaaggactgtgttgtattacatagttatttcacctcagattactaccagctgtactcaacacaagtgagtacagacactggtgttgaacatgttactttcttcatctacaataaaattgttgatgagcctgaagaacatgttcaaattcacacaatcgacggtacatctggagttgttaatccagcaatggaaccaatttatgatgaaccgacgacgactactagcgtgcctttgtaagcacaagctgatgagtacgaacttatgtactcattcgtttcggaagagacaggtacgttaatagttaatagcgtacttctttttcttgcttttgtggtattcttgctagtcacactagccatccttactgcgcttcgattgtgtgcgtactgctgcaatattgttaacgtgagtcttgtaaaaccttctttttac

SEQ ID NO: 54 - DNA, 2870 bp, Coronavirus
gtttactctcgtgttaaaaatctgaattcttctagagttcctgatcttttggtctaaacgaactaaatattatattagtctttctgtttggaactttaattttagccatgtcaggtgacaacggtaccattaccgttgaagagcttaaaaagctcttagaacaatggaacctagtaataggattcttgtttcttacatggatttgtttgttacaatttgcctatgccaacaggaataggtttttgtacataattaagttaattttcctctggctgctttggccagtaactttagcttgctttgtgcttgctgctgtttacagaataaactggatcactggtggaattgccattgcaatggcctgtcttgtaggcttgatgtggcttagctacttcattgcttctttcaggctgtttgctcgtacgcgttccatgtggtcatttaacccagaaactaacattcttttgaacgtgcctcttcatggcacaattctgaccaggccgcttctagagagtgaactcgtaattggagctgtgatccttcgtggacatcttcgtattgcaggacaccatctgggacgctgtgacatcaaggacctgcccaaagaaatcactgtagctacatcacgaacgctttcttattacaaattgggagcttcgcagcgtgtagcaggtgactcaggttttgctgcatacagtcgctacaggattggtaattacaaattaaatacagaccattccagtagcagtgacaatattgctttgcttgtacagtaagtgacaacagatgtttcatctcgttgactttcaggttactatagcagagatattattaattattatgaggacttttaaagtttccatttggaatcttgattatatcataaatctcataattaaaaatctatctaagcctccaactgagaataactgttctcaattagatgaagagcaaccaatggagattgattaaactaacatgaaaattattttcttcttggtactgataacacttgttactggcgagctttaccactaccaagagtgtataaaaggtacaactgtacttttaaaagaaccttgctcttcaggaacatatgaaggcaattcaccatttcatcctctagctgataataaatttgcactggcttgctttagcactcaatttgcttttgcttgtcctgacggtgttagacacacctttcagttacgtgcgagatcagtttcacccaaactgtttaccagacaagaggaagttcaagaattatactcacctgttttccttatcgttgcagctatagtgttcataatactttgcttcacattcaaaagaaaaatagaatgagtgaattttcattaattgacttctatttgtgcttcttagcctttctgctattccttgttttaattatgctcattatcttttggttctcactagaactgcaagatcataatgaaactttccacgcctaaacgaacatgaaatttcttgttttcttaggaattcttacaacagtagctgcattccatcaggaatgtagtttacagtcatgtgctcagcatcaaccctatgtagttgatgacccttgtccaattcacttctactcacgatggtatatcagagtgggagctagaaaatcagcacctttgattgaattgtgtgttgatgaggtaggctctaagtcacccattcaatacattgacattggtaattacacagtttcctgttctccttttacaattaattgccaggaacctaaattaggtagtctcgtagtacggtgttcgtattatgaagactttctagagtaccatgacattcgtgttgtcttagatttcatctaaacgaactaactaaaatgtctgataatggaccccaaaaccaacgtagtgcaccccgcattacatttggtggaccctcagattcaagtgacaatagcaaaaacggagagcgcaatggtgcacgacctaaacaacgtcgaccccaaggcttacccaataatactgcatcttggttcaccgctctcactcaacatggcaaggaaaaccttacgttccctcgagggcaaggtgttccaatcaacaccaatagctctaaagatgaccaaattggctactaccgtagagctaccagacgaattcgtggtggtgacggtaaaatgaaagagctcagccccagatggtatttttactatctaggaactggaccagaagctggacttccctatggtgctaacaaagaaggcatcatatgggttgcaactgagggagccttaaacacaccgaaagaccacattggcacccgcaatcctgctaacaatgctgcaatcgtgctacaacttcctcaaggaacaacattgccaaaaggcttctacgcagaagggagcagaggcggcagtcaagcttcttcacgctcctcatcacgtagtcgcaacagttcaagaaactcaactccaggcagcagtaggggaacttctcctgctagaatggctggcaatggcggtgacactgctcttgctttgctgctgctagataggttgaaccagcttgagaacaaagtatctggcaaaggccaacaacaacagggccaaactgtcactaagaaatctgctgctgaggcatctaaaaagcctcgccaaaaacgtactgctacaaaacagtacaacgtcactcaagcatttgggagacgtggtccagaacaaacccaaggaaattttggggaccaagaattaatcagacaaggaactgattacaaacattggccgcaaattgcacaatttgctccaagtgcctctgcattctttggaatgtcacgcattggcatggaagtcacaccttcgggaacatggctgacttatcatggagccatta

SEQ ID NO: 55 - DNA, 612 bp, Coronavirus
aattggatgacaaagatccacaattcaaagataacgtcatactgctgaataagcacattgacgcatacaaaacattcccaccaacagagcctaaaaaggacaaaaagaaaaaggctgatgaacttcaggctttaccgcagagacagaagaaacaacaaactgtgacccttcttcctgctgcagatttggatgaattctccaaacagttgcaacaatccatgagtggtactgattcaacccaggcttaaactcgtgcagaccacacaaggcagatgggctatataaacgttttcgcttttccgtttacgatatatagtctactcttgtgcagaatgaattctcgtaactacatagcacaagtagatgtagttaactttaatttcacatagcaatctttaatcaatgtgtaacattggggaggacttgaaagagccaccacgttttcaccgaggccacgcggagtacgatcgagggtacagccaataatgttagggagagcagcctatatggaagagccctaatgtgtaaaattaattttagtagtgctatccccatgtgattttaatagcttcaaccactcgacaagaaaaaaaaaaaaaaaaaaaaaaaaaa

SEQ ID NO: 56 - DNA, 22 bp, Artificial Sequence
  RdRP_SARSr-F2
gtgaratggtcatgtgtggcgg

SEQ ID NO: 57 - DNA, 26 bp, Artificial Sequence
  RdRP_SARSr-R1
caratgttaaasacactattagcata

SEQ ID NO: 58 - DNA, 25 bp, Artificial Sequence
  RdRP_SARSr-P2
caggtggaacctcatcaggagatgc

SEQ ID NO: 59 - DNA, 26 bp, Artificial Sequence
  RdRP_SARSr-P1
ccaggtggwacrtcatcmggtgatgc

SEQ ID NO: 60 - DNA, 26 bp, Artificial Sequence
  E_Sarbeco_P1
acactagccatccttactgcgcttcg

SEQ ID NO: 61 - DNA, 23 bp, Artificial Sequence
  2019-nCoV_N2-P
acaatttgcccccagcgcttcag

SEQ ID NO: 62 - DNA, 24 bp, Artificial Sequence
  2019-nCoV_N3-P
aycacattggcacccgcaatcctg

SEQ ID NO: 63 - DNA, 29903 bp, Coronavirus
attaaaggtttataccttcccaggtaacaaaccaaccaactttcgatctcttgtagatctgttctctaaacgaactttaaaatctgtgtggctgtcactcggctgcatgcttagtgcactcacgcagtataattaataactaattactgtcgttgacaggacacgagtaactcgtctatcttctgcaggctgcttacggtttcgtccgtgttgcagccgatcatcagcacatctaggtttcgtccgggtgtgaccgaaaggtaagatggagagccttgtccctggtttcaacgagaaaacacacgtccaactcagtttgcctgttttacaggttcgcgacgtgctcgtacgtggctttggagactccgtggaggaggtcttatcagaggcacgtcaacatcttaaagatggcacttgtggcttagtagaagttgaaaaaggcgttttgcctcaacttgaacagccctatgtgttcatcaaacgttcggatgctcgaactgcacctcatggtcatgttatggttgagctggtagcagaactcgaaggcattcagtacggtcgtagtggtgagacacttggtgtccttgtccctcatgtgggcgaaataccagtggcttaccgcaaggttcttcttcgtaagaacggtaataaaggagctggtggccatagttacggcgccgatctaaagtcatttgacttaggcgacgagcttggcactgatccttatgaagattttcaagaaaactggaacactaaacatagcagtggtgttacccgtgaactcatgcgtgagcttaacggaggggcatacactcgctatgtcgataacaacttctgtggccctgatggctaccctcttgagtgcattaaagaccttctagcacgtgctggtaaagcttcatgcactttgtccgaacaactggactttattgacactaagaggggtgtatactgctgccgtgaacatgagcatgaaattgcttggtacacggaacgttctgaaaagagctatgaattgcagacaccttttgaaattaaattggcaaagaaatttgacaccttcaatggggaatgtccaaattttgtatttcccttaaattccataatcaagactattcaaccaagggttgaaaagaaaaagcttgatggctttatgggtagaattcgatctgtctatccagttgcgtcaccaaatgaatgcaaccaaatgtgcctttcaactctcatgaagtgtgatcattgtggtgaaacttcatggcagacgggcgattttgttaaagccacttgcgaattttgtggcactgagaatttgactaaagaaggtgccactacttgtggttacttaccccaaaatgctgttgttaaaatttattgtccagcatgtcacaattcagaagtaggacctgagcatagtcttgccgaataccataatgaatctggcttgaaaaccattcttcgtaagggtggtcgcactattgcctttggaggctgtgtgttctcttatgttggttgccataacaagtgtgcctattgggttccacgtgctagcgctaacataggttgtaaccatacaggtgttgttggagaaggttccgaaggtcttaatgacaaccttcttgaaatactccaaaaagagaaagtcaacatcaatattgttggtgactttaaacttaatgaagagatcgccattattttggcatctttttctgcttccacaagtgcttttgtggaaactgtgaaaggtttggattataaagcattcaaacaaattgttgaatcctgtggtaattttaaagttacaaaaggaaaagctaaaaaaggtgcctggaatattggtgaacagaaatcaatactgagtcctctttatgcatttgcatcagaggctgctcgtgttgtacgatcaattttctcccgcactcttgaaactgctcaaaattctgtgcgtgttttacagaaggccgctataacaatactagatggaatttcacagtattcactgagactcattgatgctatgatgttcacatctgatttggctactaacaatctagttgtaatggcctacattacaggtggtgttgttcagttgacttcgcagtggctaactaacatctttggcactgtttatgaaaaactcaaacccgtccttgattggcttgaagagaagtttaaggaaggtgtagagtttcttagagacggttgggaaattgttaaatttatctcaacctgtgcttgtgaaattgtcggtggacaaattgtcacctgtgcaaaggaaattaaggagagtgttcagacattctttaagcttgtaaataaatttttggctttgtgtgctgactctatcattattggtggagctaaacttaaagccttgaatttaggtgaaacatttgtcacgcactcaaagggattgtacagaaagtgtgttaaatccagagaagaaactggcctactcatgcctctaaaagccccaaaagaaattatcttcttagagggagaaacacttcccacagaagtgttaacagaggaagttgtcttgaaaactggtgatttacaaccattagaacaacctactagtgaagctgttgaagctccattggttggtacaccagtttgtattaacgggcttatgttgctcgaaatcaaagacacagaaaagtactgtgcccttgcacctaatatgatggtaacaaacaataccttcacactcaaaggcggtgcaccaacaaaggttacttttggtgatgacactgtgatagaagtgcaaggttacaagagtgtgaatatcacttttgaacttgatgaaaggattgataaagtacttaatgagaagtgctctgcctatacagttgaactcggtacagaagtaaatgagttcgcctgtgttgtggcagatgctgtcataaaaactttgcaaccagtatctgaattacttacaccactgggcattgatttagatgagtggagtatggctacatactacttatttgatgagtctggtgagtttaaattggcttcacatatgtattgttctttctaccctccagatgaggatgaagaagaaggtgattgtgaagaagaagagtttgagccatcaactcaatatgagtatggtactgaagatgattaccaaggtaaacctttggaatttggtgccacttctgctgctcttcaacctgaagaagagcaagaagaagattggttagatgatgatagtcaacaaactgttggtcaacaagacggcagtgaggacaatcagacaactactattcaaacaattgttgaggttcaacctcaattagagatggaacttacaccagttgttcagactattgaagtgaatagttttagtggttatttaaaacttactgacaatgtatacattaaaaatgcagacattgtggaagaagctaaaaaggtaaaaccaacagtggttgttaatgcagccaatgtttaccttaaacatggaggaggtgttgcaggagccttaaataaggctactaacaatgccatgcaagttgaatctgatgattacatagctactaatggaccacttaaagtgggtggtagttgtgttttaagcggacacaatcttgctaaacactgtcttcatgttgtcggcccaaatgttaacaaaggtgaagacattcaacttcttaagagtgcttatgaaaattttaatcagcacgaagttctacttgcaccattattatcagctggtatttttggtgctgaccctatacattctttaagagtttgtgtagatactgttcgcacaaatgtctacttagctgtctttgataaaaatctctatgacaaacttgtttcaagctttttggaaatgaagagtgaaaagcaagttgaacaaaagatcgctgagattcctaaagaggaagttaagccatttataactgaaagtaaaccttcagttgaacagagaaaacaagatgataagaaaatcaaagcttgtgttgaagaagttacaacaactctggaagaaactaagttcctcacagaaaacttgttactttatattgacattaatggcaatcttcatccagattctgccactcttgttagtgacattgacatcactttcttaaagaaagatgctccatatatagtgggtgatgttgttcaagagggtgttttaactgctgtggttatacctactaaaaaggctggtggcactactgaaatgctagcgaaagctttgagaaaagtgccaacagacaattatataaccacttacccgggtcagggtttaaatggttacactgtagaggaggcaaagacagtgcttaaaaagtgtaaaagtgccttttacattctaccatctattatctctaatgagaagcaagaaattcttggaactgtttcttggaatttgcgagaaatgcttgcacatgcagaagaaacacgcaaattaatgcctgtctgtgtggaaactaaagccatagtttcaactatacagcgtaaatataagggtattaaaatacaagagggtgtggttgattatggtgctagattttacttttacaccagtaaaacaactgtagcgtcacttatcaacacacttaacgatctaaatgaaactcttgttacaatgccacttggctatgtaacacatggcttaaatttggaagaagctgctcggtatatgagatctctcaaagtgccagctacagtttctgtttcttcacctgatgctgttacagcgtataatggttatcttacttcttcttctaaaacacctgaagaacattttattgaaaccatctcacttgctggttcctataaagattggtcctattctggacaatctacacaactaggtatagaatttcttaagagaggtgataaaagtgtatattacactagtaatcctaccacattccacctagatggtgaagttatcacctttgacaatcttaagacacttctttctttgagagaagtgaggactattaaggtgtttacaacagtagacaacattaacctccacacgcaagttgtggacatgtcaatgacatatggacaacagtttggtccaacttatttggatggagctgatgttactaaaataaaacctcataattcacatgaaggtaaaacattttatgttttacctaatgatgacactctacgtgttgaggcttttgagtactaccacacaactgatcctagttttctgggtaggtacatgtcagcattaaatcacactaaaaagtggaaatacccacaagttaatggtttaacttctattaaatgggcagataacaactgttatcttgccactgcattgttaacactccaacaaatagagttgaagtttaatccacctgctctacaagatgcttattacagagcaagggctggtgaagctgctaacttttgtgcacttatcttagcctactgtaataagacagtaggtgagttaggtgatgttagagaaacaatgagttacttgtttcaacatgccaatttagattcttgcaaaagagtcttgaacgtggtgtgtaaaacttgtggacaacagcagacaacccttaagggtgtagaagctgttatgtacatgggcacactttcttatgaacaatttaagaaaggtgttcagataccttgtacgtgtggtaaacaagctacaaaatatctagtacaacaggagtcaccttttgttatgatgtcagcaccacctgctcagtatgaacttaagcatggtacatttacttgtgctagtgagtacactggtaattaccagtgtggtcactataaacatataacttctaaagaaactttgtattgcatagacggtgctttacttacaaagtcctcagaatacaaaggtcctattacggatgttttctacaaagaaaacagttacacaacaaccataaaaccagttacttataaattggatggtgttgtttgtacagaaattgaccctaagttggacaattattataagaaagacaattcttatttcacagagcaaccaattgatcttgtaccaaaccaaccatatccaaacgcaagcttcgataattttaagtttgtatgtgataatatcaaatttgctgatgatttaaaccagttaactggttataagaaacctgcttcaagagagcttaaagttacatttttccctgacttaaatggtgatgtggtggctattgattataaacactacacaccctcttttaagaaaggagctaaattgttacataaacctattgtttggcatgttaacaatgcaactaataaagccacgtataaaccaaatacctggtgtatacgttgtctttggagcacaaaaccagttgaaacatcaaattcgtttgatgtactgaagtcagaggacgcgcagggaatggataatcttgcctgcgaagatctaaaaccagtctctgaagaagtagtggaaaatcctaccatacagaaagacgttcttgagtgtaatgtgaaaactaccgaagttgtaggagacattatacttaaaccagcaaataatagtttaaaaattacagaagaggttggccacacagatctaatggctgcttatgtagacaattctagtcttactattaagaaacctaatgaattatctagagtattaggtttgaaaacccttgctactcatggtttagctgctgttaatagtgtcccttgggatactatagctaattatgctaagccttttcttaacaaagttgttagtacaactactaacatagttacacggtgtttaaaccgtgtttgtactaattatatgccttatttctttactttattgctacaattgtgtacttttactagaagtacaaattctagaattaaagcatctatgccgactactatagcaaagaatactgttaagagtgtcggtaaattttgtctagaggcttcatttaattatttgaagtcacctaatttttctaaactgataaatattataatttggtttttactattaagtgtttgcctaggttctttaatctactcaaccgctgctttaggtgttttaatgtctaatttaggcatgccttcttactgtactggttacagagaaggctatttgaactctactaatgtcactattgcaacctactgtactggttctataccttgtagtgtttgtcttagtggtttagattctttagacacctatccttctttagaaactatacaaattaccatttcatcttttaaatgggatttaactgcttttggcttagttgcagagtggtttttggcatatattcttttcactaggtttttctatgtacttggattggctgcaatcatgcaattgtttttcagctattttgcagtacattttattagtaattcttggcttatgtggttaataattaatcttgtacaaatggccccgatttcagctatggttagaatgtacatcttctttgcatcattttattatgtatggaaaagttatgtgcatgttgtagacggttgtaattcatcaacttgtatgatgtgttacaaacgtaatagagcaacaagagtcgaatgtacaactattgttaatggtgttagaaggtccttttatgtctatgctaatggaggtaaaggcttttgcaaactacacaattggaattgtgttaattgtgatacattctgtgctggtagtacatttattagtgatgaagttgcgagagacttgtcactacagtttaaaagaccaataaatcctactgaccagtcttcttacatcgttgatagtgttacagtgaagaatggttccatccatctttactttgataaagctggtcaaaagacttatgaaagacattctctctctcattttgttaacttagacaacctgagagctaataacactaaaggttcattgcctattaatgttatagtttttgatggtaaatcaaaatgtgaagaatcatctgcaaaatcagcgtctgtttactacagtcagcttatgtgtcaacctatactgttactagatcaggcattagtgtctgatgttggtgatagtgcggaagttgcagttaaaatgtttgatgcttacgttaatacgttttcatcaacttttaacgtaccaatggaaaaactcaaaacactagttgcaactgcagaagctgaacttgcaaagaatgtgtccttagacaatgtcttatctacttttatttcagcagctcggcaagggtttgttgattcagatgtagaaactaaagatgttgttgaatgtcttaaattgtcacatcaatctgacatagaagttactggcgatagttgtaataactatatgctcacctataacaaagttgaaaacatgacaccccgtgaccttggtgcttgtattgactgtagtgcgcgtcatattaatgcgcaggtagcaaaaagtcacaacattgctttgatatggaacgttaaagatttcatgtcattgtctgaacaactacgaaaacaaatacgtagtgctgctaaaaagaataacttaccttttaagttgacatgtgcaactactagacaagttgttaatgttgtaacaacaaagatagcacttaagggtggtaaaattgttaataattggttgaagcagttaattaaagttacacttgtgttcctttttgttgctgctattttctatttaataacacctgttcatgtcatgtctaaacatactgacttttcaagtgaaatcataggatacaaggctattgatggtggtgtcactcgtgacatagcatctacagatacttgttttgctaacaaacatgctgattttgacacatggtttagccagcgtggtggtagttatactaatgacaaagcttgcccattgattgctgcagtcataacaagagaagtgggttttgtcgtgcctggtttgcctggcacgatattacgcacaactaatggtgactttttgcatttcttacctagagtttttagtgcagttggtaacatctgttacacaccatcaaaacttatagagtacactgactttgcaacatcagcttgtgttttggctgctgaatgtacaatttttaaagatgcttctggtaagccagtaccatattgttatgataccaatgtactagaaggttctgttgcttatgaaagtttacgccctgacacacgttatgtgctcatggatggctctattattcaatttcctaacacctaccttgaaggttctgttagagtggtaacaacttttgattctgagtactgtaggcacggcacttgtgaaagatcagaagctggtgtttgtgtatctactagtggtagatgggtacttaacaatgattattacagatctttaccaggagttttctgtggtgtagatgctgtaaatttacttactaatatgtttacaccactaattcaacctattggtgctttggacatatcagcatctatagtagctggtggtattgtagctatcgtagtaacatgccttgcctactattttatgaggtttagaagagcttttggtgaatacagtcatgtagttgcctttaatactttactattccttatgtcattcactgtactctgtttaacaccagtttactcattcttacctggtgtttattctgttatttacttgtacttgacattttatcttactaatgatgtttcttttttagcacatattcagtggatggttatgttcacacctttagtacctttctggataacaattgcttatatcatttgtatttccacaaagcatttctattggttctttagtaattacctaaagagacgtgtagtctttaatggtgtttcctttagtacttttgaagaagctgcgctgtgcacctttttgttaaataaagaaatgtatctaaagttgcgtagtgatgtgctattacctcttacgcaatataatagatacttagctctttataataagtacaagtattttagtggagcaatggatacaactagctacagagaagctgcttgttgtcatctcgcaaaggctctcaatgacttcagtaactcaggttctgatgttctttaccaaccaccacaaacctctatcacctcagctgttttgcagagtggttttagaaaaatggcattcccatctggtaaagttgagggttgtatggtacaagtaacttgtggtacaactacacttaacggtctttggcttgatgacgtagtttactgtccaagacatgtgatctgcacctctgaagacatgcttaaccctaattatgaagatttactcattcgtaagtctaatcataatttcttggtacaggctggtaatgttcaactcagggttattggacattctatgcaaaattgtgtacttaagcttaaggttgatacagccaatcctaagacacctaagtataagtttgttcgcattcaaccaggacagactttttcagtgttagcttgttacaatggttcaccatctggtgtttaccaatgtgctatgaggcccaatttcactattaagggttcattccttaatggttcatgtggtagtgttggttttaacatagattatgactgtgtctctttttgttacatgcaccatatggaattaccaactggagttcatgctggcacagacttagaaggtaacttttatggaccttttgttgacaggcaaacagcacaagcagctggtacggacacaactattacagttaatgttttagcttggttgtacgctgctgttataaatggagacaggtggtttctcaatcgatttaccacaactcttaatgactttaaccttgtggctatgaagtacaattatgaacctctaacacaagaccatgttgacatactaggacctctttctgctcaaactggaattgccgttttagatatgtgtgcttcattaaaagaattactgcaaaatggtatgaatggacgtaccatattgggtagtgctttattagaagatgaatttacaccttttgatgttgttagacaatgctcaggtgttactttccaaagtgcagtgaaaagaacaatcaagggtacacaccactggttgttactcacaattttgacttcacttttagttttagtccagagtactcaatggtctttgttcttttttttgtatgaaaatgcctttttaccttttgctatgggtattattgctatgtctgcttttgcaatgatgtttgtcaaacataagcatgcatttctctgtttgtttttgttaccttctcttgccactgtagcttattttaatatggtctatatgcctgctagttgggtgatgcgtattatgacatggttggatatggttgatactagtttgtctggttttaagctaaaagactgtgttatgtatgcatcagctgtagtgttactaatccttatgacagcaagaactgtgtatgatgatggtgctaggagagtgtggacacttatgaatgtcttgacactcgtttataaagtttattatggtaatgctttagatcaagccatttccatgtgggctcttataatctctgttacttctaactactcaggtgtagttacaactgtcatgtttttggccagaggtattgtttttatgtgtgttgagtattgccctattttcttcataactggtaatacacttcagtgtataatgctagtttattgtttcttaggctatttttgtacttgttactttggcctcttttgtttactcaaccgctactttagactgactcttggtgtttatgattacttagtttctacacaggagtttagatatatgaattcacagggactactcccacccaagaatagcatagatgccttcaaactcaacattaaattgttgggtgttggtggcaaaccttgtatcaaagtagccactgtacagtctaaaatgtcagatgtaaagtgcacatcagtagtcttactctcagttttgcaacaactcagagtagaatcatcatctaaattgtgggctcaatgtgtccagttacacaatgacattctcttagctaaagatactactgaagcctttgaaaaaatggtttcactactttctgttttgctttccatgcagggtgctgtagacataaacaagctttgtgaagaaatgctggacaacagggcaaccttacaagctatagcctcagagtttagttcccttccatcatatgcagcttttgctactgctcaagaagcttatgagcaggctgttgctaatggtgattctgaagttgttcttaaaaagttgaagaagtctttgaatgtggctaaatctgaatttgaccgtgatgcagccatgcaacgtaagttggaaaagatggctgatcaagctatgacccaaatgtataaacaggctagatctgaggacaagagggcaaaagttactagtgctatgcagacaatgcttttcactatgcttagaaagttggataatgatgcactcaacaacattatcaacaatgcaagagatggttgtgttcccttgaacataatacctcttacaacagcagccaaactaatggttgtcataccagactataacacatataaaaatacgtgtgatggtacaacatttacttatgcatcagcattgtgggaaatccaacaggttgtagatgcagatagtaaaattgttcaacttagtgaaattagtatggacaattcacctaatttagcatggcctcttattgtaacagctttaagggccaattctgctgtcaaattacagaataatgagcttagtcctgttgcactacgacagatgtcttgtgctgccggtactacacaaactgcttgcactgatgacaatgcgttagcttactacaacacaacaaagggaggtaggtttgtacttgcactgttatccgatttacaggatttgaaatgggctagattccctaagagtgatggaactggtactatctatacagaactggaaccaccttgtaggtttgttacagacacacctaaaggtcctaaagtgaagtatttatactttattaaaggattaaacaacctaaatagaggtatggtacttggtagtttagctgccacagtacgtctacaagctggtaatgcaacagaagtgcctgccaattcaactgtattatctttctgtgcttttgctgtagatgctgctaaagcttacaaagattatctagctagtgggggacaaccaatcactaattgtgttaagatgttgtgtacacacactggtactggtcaggcaataacagttacaccggaagccaatatggatcaagaatcctttggtggtgcatcgtgttgtctgtactgccgttgccacatagatcatccaaatcctaaaggattttgtgacttaaaaggtaagtatgtacaaatacctacaacttgtgctaatgaccctgtgggttttacacttaaaaacacagtctgtaccgtctgcggtatgtggaaaggttatggctgtagttgtgatcaactccgcgaacccatgcttcagtcagctgatgcacaatcgtttttaaacgggtttgcggtgtaagtgcagcccgtcttacaccgtgcggcacaggcactagtactgatgtcgtatacagggcttttgacatctacaatgataaagtagctggttttgctaaattcctaaaaactaattgttgtcgcttccaagaaaaggacgaagatgacaatttaattgattcttactttgtagttaagagacacactttctctaactaccaacatgaagaaacaatttataatttacttaaggattgtccagctgttgctaaacatgacttctttaagtttagaatagacggtgacatggtaccacatatatcacgtcaacgtcttactaaatacacaatggcagacctcgtctatgctttaaggcattttgatgaaggtaattgtgacacattaaaagaaatacttgtcacatacaattgttgtgatgatgattatttcaataaaaaggactggtatgattttgtagaaaacccagatatattacgcgtatacgccaacttaggtgaacgtgtacgccaagctttgttaaaaacagtacaattctgtgatgccatgcgaaatgctggtattgttggtgtactgacattagataatcaagatctcaatggtaactggtatgatttcggtgatttcatacaaaccacgccaggtagtggagttcctgttgtagattcttattattcattgttaatgcctatattaaccttgaccagggctttaactgcagagtcacatgttgacactgacttaacaaagccttacattaagtgggatttgttaaaatatgacttcacggaagagaggttaaaactctttgaccgttattttaaatattgggatcagacataccacccaaattgtgttaactgtttggatgacagatgcattctgcattgtgcaaactttaatgttttattctctacagtgttcccacctacaagttttggaccactagtgagaaaaatatttgttgatggtgttccatttgtagtttcaactggataccacttcagagagctaggtgttgtacataatcaggatgtaaacttacatagctctagacttagttttaaggaattacttgtgtatgctgctgaccctgctatgcacgctgcttctggtaatctattactagataaacgcactacgtgcttttcagtagctgcacttactaacaatgttgcttttcaaactgtcaaacccggtaattttaacaaagacttctatgactttgctgtgtctaagggtttctttaaggaaggaagttctgttgaattaaaacacttcttctttgctcaggatggtaatgctgctatcagcgattatgactactatcgttataatctaccaacaatgtgtgatatcagacaactactatttgtagttgaagttgttgataagtactttgattgttacgatggtggctgtattaatgctaaccaagtcatcgtcaacaacctagacaaatcagctggttttccatttaataaatggggtaaggctagactttattatgattcaatgagttatgaggatcaagatgcacttttcgcatatacaaaacgtaatgtcatccctactataactcaaatgaatcttaagtatgccattagtgcaaagaatagagctcgcaccgtagctggtgtctctatctgtagtactatgaccaatagacagtttcatcaaaaattattgaaatcaatagccgccactagaggagctactgtagtaattggaacaagcaaattctatggtggttggcacaacatgttaaaaactgtttatagtgatgtagaaaaccctcaccttatgggttgggattatcctaaatgtgatagagccatgcctaacatgcttagaattatggcctcacttgttcttgctcgcaaacatacaacgtgttgtagcttgtcacaccgtttctatagattagctaatgagtgtgctcaagtattgagtgaaatggtcatgtgtggcggttcactatatgttaaaccaggtggaacctcatcaggagatgccacaactgcttatgctaatagtgtttttaacatttgtcaagctgtcacggccaatgttaatgcacttttatctactgatggtaacaaaattgccgataagtatgtccgcaatttacaacacagactttatgagtgtctctatagaaatagagatgttgacacagactttgtgaatgagttttacgcatatttgcgtaaacatttctcaatgatgatactctctgacgatgctgttgtgtgtttcaatagcacttatgcatctcaaggtctagtggctagcataaagaactttaagtcagttctttattatcaaaacaatgtttttatgtctgaagcaaaatgttggactgagactgaccttactaaaggacctcatgaattttgctctcaacatacaatgctagttaaacagggtgatgattatgtgtaccttccttacccagatccatcaagaatcctaggggccggctgttttgtagatgatatcgtaaaaacagatggtacacttatgattgaacggttcgtgtctttagctatagatgcttacccacttactaaacatcctaatcaggagtatgctgatgtctttcatttgtacttacaatacataagaaagctacatgatgagttaacaggacacatgttagacatgtattctgttatgcttactaatgataacacttcaaggtattgggaacctgagttttatgaggctatgtacacaccgcatacagtcttacaggctgttggggcttgtgttctttgcaattcacagacttcattaagatgtggtgcttgcatacgtagaccattcttatgttgtaaatgctgttacgaccatgtcatatcaacatcacataaattagtcttgtctgttaatccgtatgtttgcaatgctccaggttgtgatgtcacagatgtgactcaactttacttaggaggtatgagctattattgtaaatcacataaaccacccattagttttccattgtgtgctaatggacaagtttttggtttatataaaaatacatgtgttggtagcgataatgttactgactttaatgcaattgcaacatgtgactggacaaatgctggtgattacattttagctaacacctgtactgaaagactcaagctttttgcagcagaaacgctcaaagctactgaggagacatttaaactgtcttatggtattgctactgtacgtgaagtgctgtctgacagagaattacatctttcatgggaagttggtaaacctagaccaccacttaaccgaaattatgtctttactggttatcgtgtaactaaaaacagtaaagtacaaataggagagtacacctttgaaaaaggtgactatggtgatgctgttgtttaccgaggtacaacaacttacaaattaaatgttggtgattattttgtgctgacatcacatacagtaatgccattaagtgcacctacactagtgccacaagagcactatgttagaattactggcttatacccaacactcaatatctcagatgagttttctagcaatgttgcaaattatcaaaaggttggtatgcaaaagtattctacactccagggaccacctggtactggtaagagtcattttgctattggcctagctctctactacccttctgctcgcatagtgtatacagcttgctctcatgccgctgttgatgcactatgtgagaaggcattaaaatatttgcctatagataaatgtagtagaattatacctgcacgtgctcgtgtagagtgttttgataaattcaaagtgaattcaacattagaacagtatgtcttttgtactgtaaatgcattgcctgagacgacagcagatatagttgtctttgatgaaatttcaatggccacaaattatgatttgagtgttgtcaatgccagattacgtgctaagcactatgtgtacattggcgaccctgctcaattacctgcaccacgcacattgctaactaagggcacactagaaccagaatatttcaattcagtgtgtagacttatgaaaactataggtccagacatgttcctcggaacttgtcggcgttgtcctgctgaaattgttgacactgtgagtgctttggtttatgataataagcttaaagcacataaagacaaatcagctcaatgctttaaaatgttttataagggtgttatcacgcatgatgtttcatctgcaattaacaggccacaaataggcgtggtaagagaattccttacacgtaaccctgcttggagaaaagctgtctttatttcaccttataattcacagaatgctgtagcctcaaagattttgggactaccaactcaaactgttgattcatcacagggctcagaatatgactatgtcatattcactcaaaccactgaaacagctcactcttgtaatgtaaacagatttaatgttgctattaccagagcaaaagtaggcatactttgcataatgtctgatagagacctttatgacaagttgcaatttacaagtcttgaaattccacgtaggaatgtggcaactttacaagctgaaaatgtaacaggactctttaaagattgtagtaaggtaatcactgggttacatcctacacaggcacctacacacctcagtgttgacactaaattcaaaactgaaggtttatgtgttgacatacctggcatacctaaggacatgacctatagaagactcatctctatgatgggttttaaaatgaattatcaagttaatggttaccctaacatgtttatcacccgcgaagaagctataagacatgtacgtgcatggattggcttcgatgtcgaggggtgtcatgctactagagaagctgttggtaccaatttacctttacagctaggtttttctacaggtgttaacctagttgctgtacctacaggttatgttgatacacctaataatacagatttttccagagttagtgctaaaccaccgcctggagatcaatttaaacacctcataccacttatgtacaaaggacttccttggaatgtagtgcgtataaagattgtacaaatgttaagtgacacacttaaaaatctctctgacagagtcgtatttgtcttatgggcacatggctttgagttgacatctatgaagtattttgtgaaaataggacctgagcgcacctgttgtctatgtgatagacgtgccacatgcttttccactgcttcagacacttatgcctgttggcatcattctattggatttgattacgtctataatccgtttatgattgatgttcaacaatggggttttacaggtaacctacaaagcaaccatgatctgtattgtcaagtccatggtaatgcacatgtagctagttgtgatgcaatcatgactaggtgtctagctgtccacgagtgctttgttaagcgtgttgactggactattgaatatcctataattggtgatgaactgaagattaatgcggcttgtagaaaggttcaacacatggttgttaaagctgcattattagcagacaaattcccagttcttcacgacattggtaaccctaaagctattaagtgtgtacctcaagctgatgtagaatggaagttctatgatgcacagccttgtagtgacaaagcttataaaatagaagaattattctattcttatgccacacattctgacaaattcacagatggtgtatgcctattttggaattgcaatgtcgatagatatcctgctaattccattgtttgtagatttgacactagagtgctatctaaccttaacttgcctggttgtgatggtggcagtttgtatgtaaataaacatgcattccacacaccagcttttgataaaagtgcttttgttaatttaaaacaattaccatttttctattactctgacagtccatgtgagtctcatggaaaacaagtagtgtcagatatagattatgtaccactaaagtctgctacgtgtataacacgttgcaatttaggtggtgctgtctgtagacatcatgctaatgagtacagattgtatctcgatgcttataacatgatgatctcagctggctttagcttgtgggtttacaaacaatttgatacttataacctctggaacacttttacaagacttcagagtttagaaaatgtggcttttaatgttgtaaataagggacactttgatggacaacagggtgaagtaccagtttctatcattaataacactgtttacacaaaagttgatggtgttgatgtagaattgtttgaaaataaaacaacattacctgttaatgtagcatttgagctttgggctaagcgcaacattaaaccagtaccagaggtgaaaatactcaataatttgggtgtggacattgctgctaatactgtgatctgggactacaaaagagatgctccagcacatatatctactattggtgtttgttctatgactgacatagccaagaaaccaactgaaacgatttgtgcaccactcactgtcttttttgatggtagagttgatggtcaagtagacttatttagaaatgcccgtaatggtgttcttattacagaaggtagtgttaaaggtttacaaccatctgtaggtcccaaacaagctagtcttaatggagtcacattaattggagaagccgtaaaaacacagttcaattattataagaaagttgatggtgttgtccaacaattacctgaaacttactttactcagagtagaaatttacaagaatttaaacccaggagtcaaatggaaattgatttcttagaattagctatggatgaattcattgaacggtataaattagaaggctatgccttcgaacatatcgtttatggagattttagtcatagtcagttaggtggtttacatctactgattggactagctaaacgttttaaggaatcaccttttgaattagaagattttattcctatggacagtacagttaaaaactatttcataacagatgcgcaaacaggttcatctaagtgtgtgtgttctgttattgatttattacttgatgattttgttgaaataataaaatcccaagatttatctgtagtttctaaggttgtcaaagtgactattgactatacagaaatttcatttatgctttggtgtaaagatggccatgtagaaacattttacccaaaattacaatctagtcaagcgtggcaaccgggtgttgctatgcctaatctttacaaaatgcaaagaatgctattagaaaagtgtgaccttcaaaattatggtgatagtgcaacattacctaaaggcataatgatgaatgtcgcaaaatatactcaactgtgtcaatatttaaacacattaacattagctgtaccctataatatgagagttatacattttggtgctggttctgataaaggagttgcaccaggtacagctgttttaagacagtggttgcctacgggtacgctgcttgtcgattcagatcttaatgactttgtctctgatgcagattcaactttgattggtgattgtgcaactgtacatacagctaataaatgggatctcattattagtgatatgtacgaccctaagactaaaaatgttacaaaagaaaatgactctaaagagggttttttcacttacatttgtgggtttatacaacaaaagctagctcttggaggttccgtggctataaagataacagaacattcttggaatgctgatctttataagctcatgggacacttcgcatggtggacagcctttgttactaatgtgaatgcgtcatcatctgaagcatttttaattggatgtaattatcttggcaaaccacgcgaacaaatagatggttatgtcatgcatgcaaattacatattttggaggaatacaaatccaattcagttgtcttcctattctttatttgacatgagtaaatttccccttaaattaaggggtactgctgttatgtctttaaaagaaggtcaaatcaatgatatgattttatctcttcttagtaaaggtagacttataattagagaaaacaacagagttgttatttctagtgatgttcttgttaacaactaaacgaacaatgtttgtttttcttgttttattgccactagtctctagtcagtgtgttaatcttacaaccagaactcaattaccccctgcatacactaattctttcacacgtggtgtttattaccctgacaaagttttcagatcctcagttttacattcaactcaggacttgttcttacctttcttttccaatgttacttggttccatgctatacatgtctctgggaccaatggtactaagaggtttgataaccctgtcctaccatttaatgatggtgtttattttgcttccactgagaagtctaacataataagaggctggatttttggtactactttagattcgaagacccagtccctacttattgttaataacgctactaatgttgttattaaagtctgtgaatttcaattttgtaatgatccatttttgggtgtttattaccacaaaaacaacaaaagttggatggaaagtgagttcagagtttattctagtgcgaataattgcacttttgaatatgtctctcagccttttcttatggaccttgaaggaaaacagggtaatttcaaaaatcttagggaatttgtgtttaagaatattgatggttattttaaaatatattctaagcacacgcctattaatttagtgcgtgatctccctcagggtttttcggctttagaaccattggtagatttgccaataggtattaacatcactaggtttcaaactttacttgctttacatagaagttatttgactcctggtgattcttcttcaggttggacagctggtgctgcagcttattatgtgggttatcttcaacctaggacttttctattaaaatataatgaaaatggaaccattacagatgctgtagactgtgcacttgaccctctctcagaaacaaagtgtacgttgaaatccttcactgtagaaaaaggaatctatcaaacttctaactttagagtccaaccaacagaatctattgttagatttcctaatattacaaacttgtgcccttttggtgaagtttttaacgccaccagatttgcatctgtttatgcttggaacaggaagagaatcagcaactgtgttgctgattattctgtcctatataattccgcatcattttccacttttaagtgttatggagtgtctcctactaaattaaatgatctctgctttactaatgtctatgcagattcatttgtaattagaggtgatgaagtcagacaaatcgctccagggcaaactggaaagattgctgattataattataaattaccagatgattttacaggctgcgttatagcttggaattctaacaatcttgattctaaggttggtggtaattataattacctgtatagattgtttaggaagtctaatctcaaaccttttgagagagatatttcaactgaaatctatcaggccggtagcacaccttgtaatggtgttgaaggttttaattgttactttcctttacaatcatatggtttccaacccactaatggtgttggttaccaaccatacagagtagtagtactttcttttgaacttctacatgcaccagcaactgtttgtggacctaaaaagtctactaatttggttaaaaacaaatgtgtcaatttcaacttcaatggtttaacaggcacaggtgttcttactgagtctaacaaaaagtttctgcctttccaacaatttggcagagacattgctgacactactgatgctgtccgtgatccacagacacttgagattcttgacattacaccatgttcttttggtggtgtcagtgttataacaccaggaacaaatacttctaaccaggttgctgttctttatcaggatgttaactgcacagaagtccctgttgctattcatgcagatcaacttactcctacttggcgtgtttattctacaggttctaatgtttttcaaacacgtgcaggctgtttaataggggctgaacatgtcaacaactcatatgagtgtgacatacccattggtgcaggtatatgcgctagttatcagactcagactaattctcctcggcgggcacgtagtgtagctagtcaatccatcattgcctacactatgtcacttggtgcagaaaattcagttgcttactctaataactctattgccatacccacaaattttactattagtgttaccacagaaattctaccagtgtctatgaccaagacatcagtagattgtacaatgtacatttgtggtgattcaactgaatgcagcaatcttttgttgcaatatggcagtttttgtacacaattaaaccgtgctttaactggaatagctgttgaacaagacaaaaacacccaagaagtttttgcacaagtcaaacaaatttacaaaacaccaccaattaaagattttggtggttttaatttttcacaaatattaccagatccatcaaaaccaagcaagaggtcatttattgaagatctacttttcaacaaagtgacacttgcagatgctggcttcatcaaacaatatggtgattgccttggtgatattgctgctagagacctcatttgtgcacaaaagtttaacggccttactgttttgccacctttgctcacagatgaaatgattgctcaatacacttctgcactgttagcgggtacaatcacttctggttggacctttggtgcaggtgctgcattacaaataccatttgctatgcaaatggcttataggtttaatggtattggagttacacagaatgttctctatgagaaccaaaaattgattgccaaccaatttaatagtgctattggcaaaattcaagactcactttcttccacagcaagtgcacttggaaaacttcaagatgtggtcaaccaaaatgcacaagctttaaacacgcttgttaaacaacttagctccaattttggtgcaatttcaagtgttttaaatgatatcctttcacgtcttgacaaagttgaggctgaagtgcaaattgataggttgatcacaggcagacttcaaagtttgcagacatatgtgactcaacaattaattagagctgcagaaatcagagcttctgctaatcttgctgctactaaaatgtcagagtgtgtacttggacaatcaaaaagagttgatttttgtggaaagggctatcatcttatgtccttccctcagtcagcacctcatggtgtagtcttcttgcatgtgacttatgtccctgcacaagaaaagaacttcacaactgctcctgccatttgtcatgatggaaaagcacactttcctcgtgaaggtgtctttgtttcaaatggcacacactggtttgtaacacaaaggaatttttatgaaccacaaatcattactacagacaacacatttgtgtctggtaactgtgatgttgtaataggaattgtcaacaacacagtttatgatcctttgcaacctgaattagactcattcaaggaggagttagataaatattttaagaatcatacatcaccagatgttgatttaggtgacatctctggcattaatgcttcagttgtaaacattcaaaaagaaattgaccgcctcaatgaggttgccaagaatttaaatgaatctctcatcgatctccaagaacttggaaagtatgagcagtatataaaatggccatggtacatttggctaggttttatagctggcttgattgccatagtaatggtgacaattatgctttgctgtatgaccagttgctgtagttgtctcaagggctgttgttcttgtggatcctgctgcaaatttgatgaagacgactctgagccagtgctcaaaggagtcaaattacattacacataaacgaacttatggatttgtttatgagaatcttcacaattggaactgtaactttgaagcaaggtgaaatcaaggatgctactccttcagattttgttcgcgctactgcaacgataccgatacaagcctcactccctttcggatggcttattgttggcgttgcacttcttgctgtttttcagagcgcttccaaaatcataaccctcaaaaagagatggcaactagcactctccaagggtgttcactttgtttgcaacttgctgttgttgtttgtaacagtttactcacaccttttgctcgttgctgctggccttgaagccccttttctctatctttatgctttagtctacttcttgcagagtataaactttgtaagaataataatgaggctttggctttgctggaaatgccgttccaaaaacccattactttatgatgccaactattttctttgctggcatactaattgttacgactattgtataccttacaatagtgtaacttcttcaattgtcattacttcaggtgatggcacaacaagtcctatttctgaacatgactaccagattggtggttatactgaaaaatgggaatctggagtaaaagactgtgttgtattacacagttacttcacttcagactattaccagctgtactcaactcaattgagtacagacactggtgttgaacatgttaccttcttcatctacaataaaattgttgatgagcctgaagaacatgtccaaattcacacaatcgacggttcatccggagttgttaatccagtaatggaaccaatttatgatgaaccgacgacgactactagcgtgcctttgtaagcacaagctgatgagtacgaacttatgtactcattcgtttcggaagagacaggtacgttaatagttaatagcgtacttctttttcttgctttcgtggtattcttgctagttacactagccatccttactgcgcttcgattgtgtgcgtactgctgcaatattgttaacgtgagtcttgtaaaaccttctttttacgtttactctcgtgttaaaaatctgaattcttctagagttcctgatcttctggtctaaacgaactaaatattatattagtttttctgtttggaactttaattttagccatggcagattccaacggtactattaccgttgaagagcttaaaaagctccttgaacaatggaacctagtaataggtttcctattccttacatggatttgtcttctacaatttgcctatgccaacaggaataggtttttgtatataattaagttaattttcctctggctgttatggccagtaactttagcttgttttgtgcttgctgctgtttacagaataaattggatcaccggtggaattgctatcgcaatggcttgtcttgtaggcttgatgtggctcagctacttcattgcttctttcagactgtttgcgcgtacgcgttccatgtggtcattcaatccagaaactaacattcttctcaacgtgccactccatggcactattctgaccagaccgcttctagaaagtgaactcgtaatcggagctgtgatccttcgtggacatcttcgtattgctggacaccatctaggacgctgtgacatcaaggacctgcctaaagaaatcactgttgctacatcacgaacgctttcttattacaaattgggagcttcgcagcgtgtagcaggtgactcaggttttgctgcatacagtcgctacaggattggcaactataaattaaacacagaccattccagtagcagtgacaatattgctttgcttgtacagtaagtgacaacagatgtttcatctcgttgactttcaggttactatagcagagatattactaattattatgaggacttttaaagtttccatttggaatcttgattacatcataaacctcataattaaaaatttatctaagtcactaactgagaataaatattctcaattagatgaagagcaaccaatggagattgattaaacgaacatgaaaattattcttttcttggcactgataacactcgctacttgtgagctttatcactaccaagagtgtgttagaggtacaacagtacttttaaaagaaccttgctcttctggaacatacgagggcaattcaccatttcatcctctagctgataacaaatttgcactgacttgctttagcactcaatttgcttttgcttgtcctgacggcgtaaaacacgtctatcagttacgtgccagatcagtttcacctaaactgttcatcagacaagaggaagttcaagaactttactctccaatttttcttattgttgcggcaatagtgtttataacactttgcttcacactcaaaagaaagacagaatgattgaactttcattaattgacttctatttgtgctttttagcctttctgctattccttgttttaattatgcttattatcttttggttctcacttgaactgcaagatcataatgaaacttgtcacgcctaaacgaacatgaaatttcttgttttcttaggaatcatcacaactgtagctgcatttcaccaagaatgtagtttacagtcatgtactcaacatcaaccatatgtagttgatgacccgtgtcctattcacttctattctaaatggtatattagagtaggagctagaaaatcagcacctttaattgaattgtgcgtggatgaggctggttctaaatcacccattcagtacatcgatatcggtaattatacagtttcctgtttaccttttacaattaattgccaggaacctaaattgggtagtcttgtagtgcgttgttcgttctatgaagactttttagagtatcatgacgttcgtgttgttttagatttcatctaaacgaacaaactaaaatgtctgataatggaccccaaaatcagcgaaatgcaccccgcattacgtttggtggaccctcagattcaactggcagtaaccagaatggagaacgcagtggggcgcgatcaaaacaacgtcggccccaaggtttacccaataatactgcgtcttggttcaccgctctcactcaacatggcaaggaagaccttaaattccctcgaggacaaggcgttccaattaacaccaatagcagtccagatgaccaaattggctactaccgaagagctaccagacgaattcgtggtggtgacggtaaaatgaaagatctcagtccaagatggtatttctactacctaggaactgggccagaagctggacttccctatggtgctaacaaagacggcatcatatgggttgcaactgagggagccttgaatacaccaaaagatcacattggcacccgcaatcctgctaacaatgctgcaatcgtgctacaacttcctcaaggaacaacattgccaaaaggcttctacgcagaagggagcagaggcggcagtcaagcctcttctcgttcctcatcacgtagtcgcaacagttcaagaaattcaactccaggcagcagtaggggaacttctcctgctagaatggctggcaatggcggtgatgctgctcttgctttgctgctgcttgacagattgaaccagcttgagagcaaaatgtctggtaaaggccaacaacaacaaggccaaactgtcactaagaaatctgctgctgaggcttctaagaagcctcggcaaaaacgtactgccactaaagcatacaatgtaacacaagctttcggcagacgtggtccagaacaaacccaaggaaattttggggaccaggaactaatcagacaaggaactgattacaaacattggccgcaaattgcacaatttgcccccagcgcttcagcgttcttcggaatgtcgcgcattggcatggaagtcacaccttcgggaacgtggttgacctacacaggtgccatcaaattggatgacaaagatccaaatttcaaagatcaagtcattttgctgaataagcatattgacgcatacaaaacattcccaccaacagagcctaaaaaggacaaaaagaagaaggctgatgaaactcaagccttaccgcagagacagaagaaacagcaaactgtgactcttcttcctgctgcagatttggatgatttctccaaacaattgcaacaatccatgagcagtgctgactcaactcaggcctaaactcatgcagaccacacaaggcagatgggctatataaacgttttcgcttttccgtttacgatatatagtctactcttgtgcagaatgaattctcgtaactacatagcacaagtagatgtagttaactttaatctcacatagcaatctttaatcagtgtgtaacattagggaggacttgaaagagccaccacattttcaccgaggccacgcggagtacgatcgagtgtacagtgaacaatgctagggagagctgcctatatggaagagccctaatgtgtaaaattaattttagtagtgctatccccatgtgattttaatagcttcttaggagaatgacaaaaaaaaaaaaaaaaaaaaaaaaaaaaaaaaa